European Patent Application EP 4 151 235 A1, published March 22, 2023. Title: ANTIBODY DRUG CONJUGATE, PREPARATION METHOD THEREFOR AND USE THEREOF. Applicant: SICHUAN KELUN-BIOTECH BIOPHARMACEUTICAL CO., LTD. Application 21804105.1. The sequence listing filed with the application follows.

SEQUENCE LISTING (24 sequences)

SEQ ID NO: 1 - protein, 8 aa, artificial
  IMGT 2C6.9 CDR-H1
GFSLTRYG

SEQ ID NO: 2 - protein, 7 aa, artificial
  IMGT 2C6.9 CDR-H2
IWGDGNT

SEQ ID NO: 3 - protein, 11 aa, artificial
  IMGT 2C6.9 CDR-H3
ARVNFGNALDY

SEQ ID NO: 4 - protein, 12 aa, artificial
  IMGT 2C6.9 CDR-L1
QSLLNSGNQKNY

SEQ ID NO: 5 - protein, 3 aa, artificial
  IMGT 2C6.9 CDR-L2
WAS

SEQ ID NO: 6 - protein, 9 aa, artificial
  IMGT 2C6.9 CDR-L3
QNDFIFPLT

SEQ ID NO: 7 - protein, 10 aa, artificial
  AbM 2C6.9 CDR-H1
GFSLTRYGVS

SEQ ID NO: 8 - protein, 9 aa, artificial
  AbM 2C6.9 CDR-H2
VIWGDGNTN

SEQ ID NO: 9 - protein, 9 aa, artificial
  AbM 2C6.9 CDR-H3
VNFGNALDY

SEQ ID NO: 10 - protein, 17 aa, artificial
  AbM 2C6.9 CDR-L1
KSSQSLLNSGNQKNYLT

SEQ ID NO: 11 - protein, 7 aa, artificial
  AbM 2C6.9 CDR-L2
WASTRDS

SEQ ID NO: 12 - protein, 9 aa, artificial
  AbM 2C6.9 CDR-L3
QNDFIFPLT

SEQ ID NO: 13 - protein, 117 aa, artificial
  heavy chain variable region of humanized antibody 2C6.9-hz11
QVQLQESGPGLVKPSETLSLTCTVSGFSLTRYGVSWIRQPPGKGLEWIGVIWGDGNTNYNPSLKSRVTISKDSSKSQVSLKLSSVTAADTAVYYCARVNFGNALDYWGQGTLVTVSS

SEQ ID NO: 14 - protein, 117 aa, ÈË¹¤ÐòÁÐ
  heavy chain variable region of humanized antibody 2C6.9-hz21
QVQLQESGPGLVKPSETLSLTCTVSGFSLTRYGVSWIRQPPGKGLEWIGVIWGEGNTNYNPSLKSRVTISKDSSKSQVSLKLSSVTAADTAVYYCARVNFGNALDYWGQGTLVTVSS

SEQ ID NO: 15 - protein, 113 aa, artificial
  light chain variable region of humanized antibody 2C6.9-hz11/2C6.9-hz21
DIVMTQSPDSLAVSLGERATINCKSSQSLLNSGNQKNYLTWYQQKPGQPPKLLIYWASTRDSGVPDRFSGSGSGTDFTLTISSLQAEDVAVYYCQNDFIFPLTFGGGTKVEIK

SEQ ID NO: 16 - protein, 330 aa, artificial [sequence omitted]

SEQ ID NO: 17 - protein, 107 aa, artificial [sequence omitted]

SEQ ID NO: 18 - protein, 447 aa, artificial
  Full length amino acid sequence of heavy chain of humanized antibody 2C6.9-hz11
QVQLQESGPGLVKPSETLSLTCTVSGFSLTRYGVSWIRQPPGKGLEWIGVIWGDGNTNYNPSLKSRVTISKDSSKSQVSLKLSSVTAADTAVYYCARVNFGNALDYWGQGTLVTVSSASTKGPSVFPLAPSSKSTSGGTAALGCLVKDYFPEPVTVSWNSGALTSGVHTFPAVLQSSGLYSLSSVVTVPSSSLGTQTYICNVNHKPSNTKVDKKVEPKSCDKTHTCPPCPAPELLGGPSVFLFPPKPKDTLMISRTPEVTCVVVDVSHEDPEVKFNWYVDGVEVHNAKTKPREEQYNSTYRVVSVLTVLHQDWLNGKEYKCKVSNKALPAPIEKTISKAKGQPREPQVYTLPPSRDELTKNQVSLTCLVKGFYPSDIAVEWESNGQPENNYKTTPPVLDSDGSFFLYSKLTVDKSRWQQGNVFSCSVMHEALHNHYTQKSLSLSPGK

SEQ ID NO: 19 - protein, 447 aa, artificial
  Full length amino acid sequence of heavy chain of humanized antibody 2C6.9-hz21
QVQLQESGPGLVKPSETLSLTCTVSGFSLTRYGVSWIRQPPGKGLEWIGVIWGEGNTNYNPSLKSRVTISKDSSKSQVSLKLSSVTAADTAVYYCARVNFGNALDYWGQGTLVTVSSASTKGPSVFPLAPSSKSTSGGTAALGCLVKDYFPEPVTVSWNSGALTSGVHTFPAVLQSSGLYSLSSVVTVPSSSLGTQTYICNVNHKPSNTKVDKKVEPKSCDKTHTCPPCPAPELLGGPSVFLFPPKPKDTLMISRTPEVTCVVVDVSHEDPEVKFNWYVDGVEVHNAKTKPREEQYNSTYRVVSVLTVLHQDWLNGKEYKCKVSNKALPAPIEKTISKAKGQPREPQVYTLPPSRDELTKNQVSLTCLVKGFYPSDIAVEWESNGQPENNYKTTPPVLDSDGSFFLYSKLTVDKSRWQQGNVFSCSVMHEALHNHYTQKSLSLSPGK

SEQ ID NO: 20 - protein, 220 aa, aritificial
  Full length amino acid sequence of light chain of humanized antibody 2C6.9-hz11/2C6.9-hz21
DIVMTQSPDSLAVSLGERATINCKSSQSLLNSGNQKNYLTWYQQKPGQPPKLLIYWASTRDSGVPDRFSGSGSGTDFTLTISSLQAEDVAVYYCQNDFIFPLTFGGGTKVEIKRTVAAPSVFIFPPSDEQLKSGTASVVCLLNNFYPREAKVQWKVDNALQSGNSQESVTEQDSKDSTYSLSSTLTLSKADYEKHKVYACEVTHQGLSSPVTKSFNRGEC

SEQ ID NO: 21 - protein, 7 aa, artificial
  IMGT 2C6.9 CDR-H2 (after modification)
IWGEGNT

SEQ ID NO: 22 - protein, 9 aa, artificial
  AbM 2C6.9 CDR-H2 (after modification)
VIWGEGNTN

SEQ ID NO: 23 - protein, 117 aa, artificial
  heavy chain variable region of murine antibody 2C6.9M
QVQLKESGPGLVAPSQSLSITCTVSGFSLTRYGVSWVRQPPGKGLEWLGVIWGDGNTNFHSFLKSRLSISKDSSKSQVFLKLNSLQTDDTATYYCARVNFGNALDYWGQGTSVTVSS

SEQ ID NO: 24 - protein, 113 aa, artificial
  light chain variable region of murine antibody 2C6.9M
DIVMTQSPSSLTVTAGEEVTMSCKSSQSLLNSGNQKNYLTWYQQKPGQPPKLLIYWASTRDSGVPDRFTGSGSGTDFTLTISSVQSEDLAVYYCQNDFIFPLTFGAGTKLELK